European Patent Application EP 4 386 011 A1, published June 19, 2024. Title: 靶向GPC3的抗体干扰素α融合蛋白及其用途. Applicant: 上海才致药成生物科技有限公司. The sequence listing filed with the application follows.

SEQUENCE LISTING (8 sequences)

SEQ ID NO: 1 - protein, 445 aa, synthetic construct
QVQLVQSGAEVKKPGASVKVSCKASGYTFTDYEMHWVRQAPGQGLEWMGALDPKTGDTAYSQKFKGRVTLTADKSTSTAYMELSSLTSEDTAVYYCTRFYSYTYWGQGTLVTVSSASTKGPSVFPLAPSSKSTSGGTAALGCLVKDYFPEPVTVSWNSGALTSGVHTFPAVLQSSGLYSLSSVVTVPSSSLGTQTYICNVNHKPSNTKVDKKVEPKSCDKTHTCPPCPAPELLGGPSVFLFPPKPKDTLMISRTPEVTCVVVDVSHEDPEVKFNWYVDGVEVHNAKTKPREEQYNSTYRVVSVLTVLHQDWLNGKEYKCKVSNKALPAPIEKTISKAKGQPREPQVYTLPPSRDELTKNQVSLSCAVKGFYPSDIAVEWESNGQPENNYKTTPPVLDSDGSFFLVSKLTVDKSRWQQGNVFSCSVMHEALHNHYTQKSLSLSPGK

SEQ ID NO: 2 - protein, 631 aa, synthetic construct
DVVMTQSPLSLPVTPGEPASISCRSSQSLVHSNRNTYLHWYLQKPGQSPQLLIYKVSNRFSGVPDRFSGSGSGTDFTLKISRVEAEDVGVYYCSQNTHVPPTFGQGTKLEIKRTVAAPSVFIFPPSDEQLKSGTASVVCLLNNFYPREAKVQWKVDNALQSGNSQESVTEQDSKDSTYSLSSTLTLSKADYEKHKVYACEVTHQGLSSPVTKSFNRGECGGGGSGGGGSGGGGSGGGGSCDLPQTHSLGSRRTLMLLAQMRRISLFSCLKDRHDFGFPQEEFGNQFQKAETIPVLHEMIQQIFNLFSTKDSSAAWDETLLDKFYTELYQQLNDLEACVIQGVGVTETPLMKEDSILAVRKYFQRITLYLKEKKYSPCAWEVVRGEIMRSFSLSTNLQESLRSKEDKTHTCPPCPAPELLGGPSVFLFPPKPKDTLMISRTPEVTCVVVDVSHEDPEVKFNWYVDGVEVHNAKTKPREEQYNSTYRVVSVLTVLHQDWLNGKEYKCKVSNKALPAPIEKTISKAKGQPREPQVYTLPPSRDELTKNQVSLWCLVKGFYPSDIAVEWESNGQPENNYKTTPPVLDSDGSFFLYSKLTVDKSRWQQGNVFSCSVMHEALHNHYTQKSLSLSPGK

SEQ ID NO: 3 - protein, 188 aa, synthetic construct
MALTFALLVALLVLSCKSSCSVGCDLPQTHSLGSRRTLMLLAQMRRISLFSCLKDRHDFGFPQEEFGNQFQKAETIPVLHEMIQQIFNLFSTKDSSAAWDETLLDKFYTELYQQLNDLEACVIQGVGVTETPLMKEDSILAVRKYFQRITLYLKEKKYSPCAWEVVRAEIMRSFSLSTNLQESLRSKE

SEQ ID NO: 4 - protein, 165 aa, synthetic construct [sequence omitted]

SEQ ID NO: 5 - protein, 392 aa, synthetic construct
CDLPQTHSLGSRRTLMLLAQMRRISLFSCLKDRHDFGFPQEEFGNQFQKAETIPVLHEMIQQIFNLFSTKDSSAAWDETLLDKFYTELYQQLNDLEACVIQGVGVTETPLMKEDSILAVRKYFQRITLYLKEKKYSPCAWEVVRAEIMRSFSLSTNLQESLRSKEDKTHTCPPCPAPELLGGPSVFLFPPKPKDTLMISRTPEVTCVVVDVSHEDPEVKFNWYVDGVEVHNAKTKPREEQYNSTYRVVSVLTVLHQDWLNGKEYKCKVSNKALPAPIEKTISKAKGQPREPQVYTLPPSRDELTKNQVSLSCAVKGFYPSDIAVEWESNGQPENNYKTTPPVLDSDGSFFLVSKLTVDKSRWQQGNVFSCSVMHEALHNHYTQKSLSLSPGK

SEQ ID NO: 6 - protein, 445 aa, synthetic construct
QVQLVQSGAEVKKPGASVKVSCKASGYTFTDYEMHWVRQAPGQGLEWMGALDPKTGDTAYSQKFKGRVTLTADKSTSTAYMELSSLTSEDTAVYYCTRFYSYTYWGQGTLVTVSSASTKGPSVFPLAPSSKSTSGGTAALGCLVKDYFPEPVTVSWNSGALTSGVHTFPAVLQSSGLYSLSSVVTVPSSSLGTQTYICNVNHKPSNTKVDKKVEPKSCDKTHTCPPCPAPELLGGPSVFLFPPKPKDTLMISRTPEVTCVVVDVSHEDPEVKFNWYVDGVEVHNAKTKPREEQYNSTYRVVSVLTVLHQDWLNGKEYKCKVSNKALPAPIEKTISKAKGQPREPQVYTLPPSREEMTKNQVSLTCLVKGFYPSDIAVEWESNGQPENNYKTTPPVLDSDGSFFLYSKLTVDKSRWQQGNVFSCSVMHEALHNHYTQKSLSLSPGK

SEQ ID NO: 7 - protein, 219 aa, synthetic construct
DVVMTQSPLSLPVTPGEPASISCRSSQSLVHSNRNTYLHWYLQKPGQSPQLLIYKVSNRFSGVPDRFSGSGSGTDFTLKISRVEAEDVGVYYCSQNTHVPPTFGQGTKLEIKRTVAAPSVFIFPPSDEQLKSGTASVVCLLNNFYPREAKVQWKVDNALQSGNSQESVTEQDSKDSTYSLSSTLTLSKADYEKHKVYACEVTHQGLSSPVTKSFNRGEC

SEQ ID NO: 8 - protein, 17 aa, synthetic construct
MRAWIFFLLCLAGRALA